European Patent Application EP 4 397 762 A1, published July 10, 2024. Title: Anti-growth hormone antibody. Applicant: TAISHO PHARMACEUTICAL CO., LTD. The sequence listing filed with the application follows.

SEQUENCE LISTING (20 sequences)

SEQ ID NO: 1 - DNA, 414 bp, Mus musculus
  source 1..414: mol_type = other DNA
atggaatggaactgggtcgttctcttcctcctgtcattaactgcaggtgtctatgcccagggtcagatgcagcagtctggaggtgagttggtgaatcctgggtcttcagtgaagatgtcctgcaagacttctggcttcaccttcaccagtagtgaaataagttggttgaagcagaagcctggacagagtcttgagtggattgcatggatttatcctggaactggtagtagtaagtttaatcagaagttcacgggcaaggcccaactgactgcagaaacatcctccagcacagcctacatgcaactcagcagcctgacatctgaggactctgccatctattactgtgcaagacgggggttcttcggtggtagttttgactactggggccaaggcaccactctcacaatctcctca

SEQ ID NO: 2 - DNA, 390 bp, Mus musculus
  source 1..390: mol_type = other DNA
atggattttcaggtgcagattttcagcttcctgctaatcagtgcctcagtcgtaatgtccagaggacaaattgttctcgcccagtctccagcaatcatgtctgcatctctaggggaacgggtcaccatgacctgcactgccacctcaagtgtaagttccagttacttgcactggtaccagcagaagccaggatcctcccccaaactctggatttatagcacatccaacctggcttctggagtcccagctcgcttcagtggcagtgggtctgggacctcttactctctcacaatcagcagcatggaggctgaagatgctgccacttattactgccaccagtatcatcattccccacccacgttcggtgctgggaccaagctggagctgaaa

SEQ ID NO: 3 - protein, 119 aa, Mus musculus
QGQMQQSGGELVNPGSSVKMSCKTSGFTFTSSEISWLKQKPGQSLEWIAWIYPGTGSSKFNQKFTGKAQLTAETSSSTAYMQLSSLTSEDSAIYYCARRGFFGGSFDYWGQGTTLTISS

SEQ ID NO: 4 - protein, 108 aa, Mus musculus
QIVLAQSPAIMSASLGERVTMTCTATSSVSSSYLHWYQQKPGSSPKLWIYSTSNLASGVPARFSGSGSGTSYSLTISSMEAEDAATYYCHQYHHSPPTFGAGTKLELK

SEQ ID NO: 5 - protein, 5 aa, Mus musculus
SSEIS

SEQ ID NO: 6 - protein, 17 aa, Mus musculus
WIYPGTGSSKFNQKFTG

SEQ ID NO: 7 - protein, 10 aa, Mus musculus
RGFFGGSFDY

SEQ ID NO: 8 - protein, 12 aa, Mus musculus
TATSSVSSSYLH

SEQ ID NO: 9 - protein, 7 aa, Mus musculus
STSNLAS

SEQ ID NO: 10 - protein, 9 aa, Mus musculus
HQYHHSPPT

SEQ ID NO: 11 - protein, 138 aa, synthetic construct
  REGION 1..138: note = Synthetic
MEWNWVVLFLLSLTAGVYAQVQMVQSGAEVKKPGASVKVSCKASGFTFTSSEISWLRQAPGQRLEWIAWIYPGTGSSKFNQKFTGKATLTADTSASTAYMELSSLRSEDTAVYYCARRGFFGGSFDYWGQGTTVTVSS

SEQ ID NO: 12 - protein, 119 aa, synthetic construct
  REGION 1..119: note = Synthetic
QVQMVQSGAEVKKPGASVKVSCKASGFTFTSSEISWLRQAPGQRLEWIAWIYPGTGSSKFNQKFTGKATLTADTSASTAYMELSSLRSEDTAVYYCARRGFFGGSFDYWGQGTTVTVSS

SEQ ID NO: 13 - protein, 130 aa, synthetic construct
  REGION 1..130: note = Synthetic
MDFQVQIFSFLLISASVVMSRGDIQLTQSPSFLSASVGDRVTITCTATSSVSSSYLHWYQQKPGKAPKLWIYSTSNLASGVPSRFSGSGSGTEFTLTISSLQPEDFATYYCHQYHHSPPTFGGGTKVEIK

SEQ ID NO: 14 - protein, 108 aa, synthetic construct
  REGION 1..108: note = Synthetic
DIQLTQSPSFLSASVGDRVTITCTATSSVSSSYLHWYQQKPGKAPKLWIYSTSNLASGVPSRFSGSGSGTEFTLTISSLQPEDFATYYCHQYHHSPPTFGGGTKVEIK

SEQ ID NO: 15 - DNA, 414 bp, synthetic construct
  misc_feature 1..414: note = Synthetic
  source 1..414: mol_type = other DNA
atggaatggaactgggtcgtgctgttcctgctgtctctgaccgctggcgtgtacgctcaggttcagatggttcagtctggcgccgaagtgaagaaacctggcgcctctgtgaaggtgtcctgcaaggcttccggcttcacctttacctccagcgagatctcttggctgagacaggctcctggccagcggctggaatggatcgcttggatctatcctggcaccggctcctccaagttcaaccagaaattcaccggcaaagccaccctgaccgccgacacctctgcttctaccgcctacatggaactgtccagcctgagatctgaggacaccgccgtgtactactgcgccagaagaggcttcttcggcggctcctttgattactggggccagggcacaaccgtgaccgtttcttct

SEQ ID NO: 16 - DNA, 390 bp, synthetic construct
  misc_feature 1..390: note = Synthetic
  source 1..390: mol_type = other DNA
atggacttccaggtgcagatcttctccttcctgctgatctccgcctccgtggtcatgtccagaggcgacattcagctgacccagtctccatccttcctgtccgcctctgtgggcgacagagtgaccattacctgtaccgctacctcctccgtgtcctcctcttacctgcactggtatcagcagaagcccggcaaggctcccaagctgtggatctactccacctccaatctggcctctggcgtgccctctagattctccggatctggctctggaaccgagtttaccctgacaatctccagcctgcagcctgaggacttcgccacctactactgccaccagtaccaccactctccacctacctttggcggaggcaccaaggtggaaatcaag

SEQ ID NO: 17 - protein, 330 aa, synthetic construct
  REGION 1..330: note = Synthetic
ASTKGPSVFPLAPSSKSTSGGTAALGCLVKDYFPEPVTVSWNSGALTSGVHTFPAVLQSSGLYSLSSVVTVPSSSLGTQTYICNVNHKPSNTKVDKKVEPKSCDKTHTCPPCPAPELLGGPSVFLFPPKPKDTLMISRTPEVTCVVVDVSHEDPEVKFNWYVDGVEVHNAKTKPREEQYNSTYRVVSVLTVLHQDWLNGKEYKCKVSNKALPAPIEKTISKAKGQPREPQVYTLPPSRDELTKNQVSLTCLVKGFYPSDIAVEWESNGQPENNYKTTPPVLDSDGSFFLYSKLTVDKSRWQQGNVFSCSVLHEALHNHYTQKSLSLSPGK

SEQ ID NO: 18 - protein, 107 aa, Homo sapiens [sequence omitted]

SEQ ID NO: 19 - protein, 138 aa, Mus musculus
MEWNWVVLFLLSLTAGVYAQGQMQQSGGELVNPGSSVKMSCKTSGFTFTSSEISWLKQKPGQSLEWIAWIYPGTGSSKFNQKFTGKAQLTAETSSSTAYMQLSSLTSEDSAIYYCARRGFFGGSFDYWGQGTTLTISS

SEQ ID NO: 20 - protein, 130 aa, Mus musculus
MDFQVQIFSFLLISASVVMSRGQIVLAQSPAIMSASLGERVTMTCTATSSVSSSYLHWYQQKPGSSPKLWIYSTSNLASGVPARFSGSGSGTSYSLTISSMEAEDAATYYCHQYHHSPPTFGAGTKLELK